European Patent Application EP 4 306 652 A2, published January 17, 2024. Title: BISULFITE-FREE, WHOLE GENOME METHYLATION ANALYSIS. Applicant: Ludwig Institute for Cancer Research Ltd. Application WO PCT/IB2020/056435, filed July 8, 2020. The sequence listing filed with the application follows.

SEQUENCE LISTING (76 sequences)

SEQ ID NO: 1 - DNA, 12 bp, synthetic construct
  misc_feature 1..12: note = source = /note="Description of Artificial Sequence: Synthetic oligonucleotide"
  source 1..12: mol_type = other DNA
gtcgaccggatc

SEQ ID NO: 2 - DNA, 17 bp, synthetic construct
  misc_feature 1..17: note = source = /note="Description of Artificial Sequence: Synthetic oligonucleotide"
  source 1..17: mol_type = other DNA
ttggatccggtcgactt

SEQ ID NO: 3 - DNA, 20 bp, synthetic construct
  misc_feature 1..20: note = source = /note="Description of Artificial Sequence: Synthetic primer"
  source 1..20: mol_type = other DNA
cctgatgaaacaagcatgtc

SEQ ID NO: 4 - DNA, 20 bp, synthetic construct
  misc_feature 1..20: note = source = /note="Description of Artificial Sequence: Synthetic primer"
  misc_feature 1..20: note = source = /note="Description of Combined DNA/RNA Molecule: Synthetic primer"
  source 1..20: mol_type = other DNA
  misc_feature 3: note = RNA
  misc_feature 11: note = RNA
  misc_feature 19: note = RNA
cattactcacttccccactt

SEQ ID NO: 5 - DNA, 36 bp, synthetic construct
  misc_feature 1..36: note = source = /note="Description of Artificial Sequence: Synthetic oligonucleotide"
  source 1..36: mol_type = other DNA
cccgacgcatgatctgtacttgatcgaccgtgcaac

SEQ ID NO: 6 - DNA, 58 bp, synthetic construct
  misc_feature 1..58: note = source = /note="Description of Artificial Sequence: Synthetic oligonucleotide"
  source 1..58: mol_type = other DNA
aatgatacggcgaccaccgagatctacactctttccctacacgacgctcttccgatct

SEQ ID NO: 7 - DNA, 63 bp, synthetic construct
  misc_feature 1..63: note = source = /note="Description of Artificial Sequence: Synthetic oligonucleotide"
  source 1..63: mol_type = other DNA
gatcggaagagcacacgtctgaactccagtcacgccaatatctcgtatgccgtcttctgcttg

SEQ ID NO: 8 - DNA, 56 bp, synthetic construct
  misc_feature 1..56: note = source = /note="Description of Artificial Sequence: Synthetic oligonucleotide"
  misc_feature 1..56: note = source = /note="Description of Combined DNA/RNA Molecule: Synthetic oligonucleotide"
  source 1..56: mol_type = other DNA
  misc_feature 9: note = RNA
  misc_feature 20: note = RNA
  misc_feature 29: note = RNA
  misc_feature 42: note = RNA
  misc_feature 50: note = RNA
tcttccgatcgttgcacggtcgatcaagtacagatcatgcgtcgggagatcggaag

SEQ ID NO: 9 - DNA, 157 bp, synthetic construct
  misc_feature 1..157: note = source = /note="Description of Artificial Sequence: Synthetic polynucleotide"
  source 1..157: mol_type = other DNA
aatgatacggcgaccaccgagatctacactctttccctacacgacgctcttccgatctcccgacgcatgatctgtacttgatcgaccgtgcaacgatcggaagagcacacgtctgaactccagtcacgccaatatctcgtatgccgtcttctgcttg

SEQ ID NO: 10 - DNA, 21 bp, synthetic construct
  misc_feature 1..21: note = source = /note="Description of Artificial Sequence: Synthetic primer"
  source 1..21: mol_type = other DNA
aatgatacggcgaccaccgag

SEQ ID NO: 11 - DNA, 22 bp, synthetic construct
  misc_feature 1..22: note = source = /note="Description of Artificial Sequence: Synthetic primer"
  source 1..22: mol_type = other DNA
caagcagaagacggcatacgag

SEQ ID NO: 12 - DNA, 34 bp, synthetic construct
  misc_feature 1..34: note = source = /note="Description of Artificial Sequence: Synthetic oligonucleotide"
  source 1..34: mol_type = other DNA
agcagtctcgatcagctgctactgtacgtagcat

SEQ ID NO: 13 - DNA, 40 bp, synthetic construct
  misc_feature 1..40: note = source = /note="Description of Artificial Sequence: Synthetic oligonucleotide"
  source 1..40: mol_type = other DNA
aggtgcgctaagttctagatcgccaactggttgtggcctt

SEQ ID NO: 14 - DNA, 60 bp, synthetic construct
  misc_feature 1..60: note = source = /note="Description of Artificial Sequence: Synthetic oligonucleotide"
  source 1..60: mol_type = other DNA
ctatagccggcttgctctctctgcctctagcagctgctccctatagtgagtcgtattaac

SEQ ID NO: 15 - DNA, 40 bp, synthetic construct
  misc_feature 1..40: note = source = /note="Description of Artificial Sequence: Synthetic oligonucleotide"
  source 1..40: mol_type = other DNA
atctagaacttagcgcacctagatcggaagagcgtcgtgt

SEQ ID NO: 16 - DNA, 74 bp, synthetic construct
  misc_feature 1..74: note = source = /note="Description of Artificial Sequence: Synthetic oligonucleotide"
  source 1..74: mol_type = other DNA
agagagcaagccggctatagatgctacgtacagtagcagctgatcaagactgctaaggccacaaccagttggcg

SEQ ID NO: 17 - DNA, 42 bp, synthetic construct
  misc_feature 1..42: note = source = /note="Description of Artificial Sequence: Synthetic oligonucleotide"
  source 1..42: mol_type = other DNA
agacgtgtgctcttccgatcgttaatacgactcactataggg

SEQ ID NO: 18 - DNA, 255 bp, synthetic construct
  misc_feature 1..255: note = source = /note="Description of Artificial Sequence: Synthetic polynucleotide"
  source 1..255: mol_type = other DNA
aatgatacggcgaccaccgagatctacactctttccctacacgacgctcttccgatctaggtgcgctaagttctagatcgccaactggttgtggccttagcagtctcgatcagctgctactgtacgtagcatctatagccggcttgctctctctgcctctagcagctgctccctatagtgagtcgtattaacgatcggaagagcacacgtctgaactccagtcacgccaatatctcgtatgccgtcttctgcttg

SEQ ID NO: 19 - DNA, 22 bp, synthetic construct
  misc_feature 1..22: note = source = /note="Description of Artificial Sequence: Synthetic oligonucleotide"
  source 1..22: mol_type = other DNA
tgctagaggcagagagagcaag

SEQ ID NO: 20 - DNA, 17 bp, synthetic construct
  variation 9: note = /replace="DHU" or "t" or "c"
  misc_feature 1..17: note = /note="Variant nucleotides given in the sequence have no preference with respect to those in the annotations for variant positions"
  misc_feature 1..17: note = source = /note="Description of Artificial Sequence: Synthetic oligonucleotide"
  misc_feature 1..17: note = source = /note="Description of Combined DNA/RNA Molecule: Synthetic oligonucleotide"
  source 1..17: mol_type = other DNA
  misc_feature 9: note = RNA
agcagtcttgatcagct

SEQ ID NO: 21 - DNA, 17 bp, synthetic construct
  misc_feature 1..17: note = source = /note="Description of Artificial Sequence: Synthetic oligonucleotide"
  source 1..17: mol_type = other DNA
gctactgtacgtagcat

SEQ ID NO: 22 - DNA, 255 bp, synthetic construct
  variation 107: note = /replace="DHU" or "t" or "c"
  misc_feature 1..255: note = /note="Variant nucleotides given in the sequence have no preference with respect to those in the annotations for variant positions"
  misc_feature 1..255: note = source = /note="Description of Artificial Sequence: Synthetic oligonucleotide"
  misc_feature 1..255: note = source = /note="Description of Combined DNA/RNA Molecule: Synthetic oligonucleotide"
  source 1..255: mol_type = other DNA
  misc_feature 117: note = RNA
aatgatacggcgaccaccgagatctacactctttccctacacgacgctcttccgatctaggtgcgctaagttctagatcgccaactggttgtggccttagcagtcttgatcagctgctactgtacgtagcatctatagccggcttgctctctctgcctctagcagctgctccctatagtgagtcgtattaacgatcggaagagcacacgtctgaactccagtcacgccaatatctcgtatgccgtcttctgcttg

SEQ ID NO: 23 - DNA, 20 bp, synthetic construct
  misc_feature 1..20: note = source = /note="Description of Artificial Sequence: Synthetic primer"
  source 1..20: mol_type = other DNA
cacagatgtctgcctgttca

SEQ ID NO: 24 - DNA, 20 bp, synthetic construct
  misc_feature 1..20: note = source = /note="Description of Artificial Sequence: Synthetic primer"
  source 1..20: mol_type = other DNA
agggtggtgaatgtgaaacc

SEQ ID NO: 25 - DNA, 2018 bp, synthetic construct
  misc_feature 1..2018: note = source = /note="Description of Artificial Sequence: Synthetic polynucleotide"
  source 1..2018: mol_type = other DNA
cacagatgtctgcctgttcatccgcgtccagctcgttgagtttctccagaagcgttaatgtctggcttctgataaagcgggccatgttaagggcggttttttcctgtttggtcactgatgcctccgtgtaagggggatttctgttcatgggggtaatgataccgatgaaacgagagaggatgctcacgatacgggttactgatgatgaacatgcccggttactggaacgttgtgagggtaaacaactggcggtatggatgcggcgggaccagagaaaaatcactcagggtcaatgccagcgcttcgttaatacagatgtaggtgttccacagggtagccagcagcatcctgcgatgcagatccggaacataatggtgcagggcgctgacttccgcgtttccagactttacgaaacacggaaaccgaagaccattcatgttgttgctcaggtcgcagacgttttgcagcagcagtcgcttcacgttcgctcgcgtatcggtgattcattctgctaaccagtaaggcaaccccgccagcctagccgggtcctcaacgacaggagcacgatcatgcgcacccgtggggccgccatgccggcgataatggcctgcttctcgccgaaacgtttggtggcgggaccagtgacgaaggcttgagcgagggcgtgcaagattccgaataccgcaagcgacaggccgatcatcgtcgcgctccagcgaaagcggtcctcgccgaaaatgacccagagcgctgccggcacctgtcctacgagttgcatgataaagaagacagtcataagtgcggcgacgatagtcatgccccgcgcccaccggaaggagctgactgggttgaaggctctcaagggcatcggtcgagatcccggtgcctaatgagtgagctaacttacattaattgcgttgcgctcactgcccgctttccagtcgggaaacctgtcgtgccagctgcattaatgaatcggccaacgcgcggggagaggcggtttgcgtattgggcgccagggtggtttttcttttcaccagtgagacgggcaacagctgattgcccttcaccgcctggccctgagagagttgcagcaagcggtccacgctggtttgccccagcaggcgaaaatcctgtttgatggtggttaacggcgggatataacatgagctgtcttcggtatcgtcgtatcccactaccgagatatccgcaccaacgcgcagcccggactcggtaatggcgcgcattgcgcccagcgccatctgatcgttggcaaccagcatcgcagtgggaacgatgccctcattcagcatttgcatggtttgttgaaaaccggacatggcactccagtcgccttcccgttccgctatcggctgaatttgattgcgagtgagatatttatgccagccagccagacgcagacgcgccgagacagaacttaatgggcccgctaacagcgcgatttgctggtgacccaatgcgaccagatgctccacgcccagtcgcgtaccgtcttcatgggagaaaataatactgttgatgggtgtctggtcagagacatcaagaaataacgccggaacattagtgcaggcagcttccacagcaatggcatcctggtcatccagcggatagttaatgatcagcccactgacgcgttgcgcgagaagattgtgcaccgccgctttacaggcttcgacgccgcttcgttctaccatcgacaccaccacgctggcacccagttgatcggcgcgagatttaatcgccgcgacaatttgcgacggcgcgtgcagggccagactggaggtggcaacgccaatcagcaacgactgtttgcccgccagttgttgtgccacgcggttgggaatgtaattcagctccgccatcgccgcttccactttttcccgcgttttcgcagaaacgtggctggcctggttcaccacgcgggaaacggtctgataagagacaccggcatactctgcgacatcgtataacgttactggtttcacattcaccaccct

SEQ ID NO: 26 - DNA, 120 bp, synthetic construct
  misc_feature 1..120: note = source = /note="Description of Artificial Sequence: Synthetic polynucleotide"
  source 1..120: mol_type = other DNA
atactcatcattaaacttcgcccttacctaccacttcgtgtatgtagataggtagtatacaattgatatcgaaatgagtacgtagatagtagaaagtaagatggaggtgagagtgagagt

SEQ ID NO: 27 - DNA, 38 bp, synthetic construct
  misc_feature 1..38: note = source = /note="Description of Artificial Sequence: Synthetic primer"
  source 1..38: mol_type = other DNA
atactcatcattaaacttcgcccttacctaccacttcg

SEQ ID NO: 28 - DNA, 120 bp, synthetic construct
  misc_feature 1..120: note = source = /note="Description of Artificial Sequence: Synthetic polynucleotide"
  source 1..120: mol_type = other DNA
gcggcgtgatactggtcccgagcctgaagttaggcccgggatgactgacagtcttccgagaccgacgacacaggtctccctatagtgagtcgtattatggcgagagaatgaatctccatc

SEQ ID NO: 29 - DNA, 42 bp, synthetic construct
  misc_feature 1..42: note = source = /note="Description of Artificial Sequence: Synthetic primer"
  source 1..42: mol_type = other DNA
gatggagattcattctctcgccataatacgactcactatagg

SEQ ID NO: 30 - DNA, 90 bp, synthetic construct
  modified_base 50: mod_base = OTHER; note = a, c, t, g, unknown or other
  modified_base 52..53: mod_base = OTHER; note = a, c, t, g, unknown or other
  misc_feature 1..90: note = source = /note="Description of Artificial Sequence: Synthetic oligonucleotide"
  source 1..90: mol_type = other DNA
gaagatgcagaagacaggaaggatgaaacactcaggcgcacgctggcatncnngacaaaccacaagaacaggctagtgagaatgaaggga

SEQ ID NO: 31 - DNA, 90 bp, synthetic construct
  modified_base 49: mod_base = OTHER; note = a, c, t, g, unknown or other
  modified_base 51..52: mod_base = OTHER; note = a, c, t, g, unknown or other
  misc_feature 1..90: note = source = /note="Description of Artificial Sequence: Synthetic oligonucleotide"
  source 1..90: mol_type = other DNA
ccaactctgaaacccaccaacgccaacatccaccacacaacccaagatncnngaccatcttacaaacatatcccttcattctcactagcc

SEQ ID NO: 32 - DNA, 160 bp, synthetic construct
  modified_base 50: mod_base = OTHER; note = a, c, t, g, unknown or other
  modified_base 52..53: mod_base = OTHER; note = a, c, t, g, unknown or other
  modified_base 109..110: mod_base = OTHER; note = a, c, t, g, unknown or other
  modified_base 112: mod_base = OTHER; note = a, c, t, g, unknown or other
  misc_feature 1..160: note = source = /note="Description of Artificial Sequence: Synthetic polynucleotide"
  source 1..160: mol_type = other DNA
gaagatgcagaagacaggaaggatgaaacactcaggcgcacgctggcatncnngacaaaccacaagaacaggctagtgagaatgaagggatatgtttgtaagatggtcnngnatcttgggttgtgtggtggatgttggcgttggtgggtttcagagttgg

SEQ ID NO: 33 - DNA, 160 bp, synthetic construct
  modified_base 49: mod_base = OTHER; note = a, c, t, g, unknown or other
  modified_base 51..52: mod_base = OTHER; note = a, c, t, g, unknown or other
  modified_base 108..109: mod_base = OTHER; note = a, c, t, g, unknown or other
  modified_base 111: mod_base = OTHER; note = a, c, t, g, unknown or other
  misc_feature 1..160: note = source = /note="Description of Artificial Sequence: Synthetic polynucleotide"
  source 1..160: mol_type = other DNA
ccaactctgaaacccaccaacgccaacatccaccacacaacccaagatncnngaccatcttacaaacatatcccttcattctcactagcctgttcttgtggtttgtcnngnatgccagcgtgcgcctgagtgtttcatccttcctgtcttctgcatcttc

SEQ ID NO: 34 - DNA, 20 bp, synthetic construct
  misc_feature 1..20: note = source = /note="Description of Artificial Sequence: Synthetic primer"
  source 1..20: mol_type = other DNA
cattactcacttccccactt

SEQ ID NO: 35 - DNA, 20 bp, synthetic construct
  misc_feature 1..20: note = source = /note="Description of Artificial Sequence: Synthetic primer"
  source 1..20: mol_type = other DNA
gctgcagattggagccaaag

SEQ ID NO: 36 - DNA, 20 bp, synthetic construct
  misc_feature 1..20: note = source = /note="Description of Artificial Sequence: Synthetic primer"
  source 1..20: mol_type = other DNA
ttgatggtgatggtggagcc

SEQ ID NO: 37 - DNA, 22 bp, synthetic construct
  misc_feature 1..22: note = source = /note="Description of Artificial Sequence: Synthetic primer"
  source 1..22: mol_type = other DNA
tcagtgctcatggactcatact

SEQ ID NO: 38 - DNA, 23 bp, synthetic construct
  misc_feature 1..23: note = source = /note="Description of Artificial Sequence: Synthetic primer"
  source 1..23: mol_type = other DNA
ataccctgggagcaaagttgttg

SEQ ID NO: 39 - DNA, 20 bp, synthetic construct
  misc_feature 1..20: note = source = /note="Description of Artificial Sequence: Synthetic primer"
  source 1..20: mol_type = other DNA
cccactagacatgctctgcc

SEQ ID NO: 40 - DNA, 21 bp, synthetic construct
  misc_feature 1..21: note = source = /note="Description of Artificial Sequence: Synthetic primer"
  source 1..21: mol_type = other DNA
caaaatgttgcttgccttccg

SEQ ID NO: 41 - DNA, 20 bp, synthetic construct
  misc_feature 1..20: note = source = /note="Description of Artificial Sequence: Synthetic primer"
  source 1..20: mol_type = other DNA
tccctgagccctgatctagt

SEQ ID NO: 42 - DNA, 20 bp, synthetic construct
  misc_feature 1..20: note = source = /note="Description of Artificial Sequence: Synthetic primer"
  source 1..20: mol_type = other DNA
aatactggctgaccggttct

SEQ ID NO: 43 - DNA, 20 bp, synthetic construct
  misc_feature 1..20: note = source = /note="Description of Artificial Sequence: Synthetic primer"
  source 1..20: mol_type = other DNA
acaccacagcagaagagagc

SEQ ID NO: 44 - DNA, 20 bp, synthetic construct
  misc_feature 1..20: note = source = /note="Description of Artificial Sequence: Synthetic primer"
  source 1..20: mol_type = other DNA
taggattgttgcacaggcca

SEQ ID NO: 45 - DNA, 21 bp, synthetic construct
  misc_feature 1..21: note = source = /note="Description of Artificial Sequence: Synthetic primer"
  source 1..21: mol_type = other DNA
gctgagctgtatccttgaggt

SEQ ID NO: 46 - DNA, 20 bp, synthetic construct
  misc_feature 1..20: note = source = /note="Description of Artificial Sequence: Synthetic primer"
  source 1..20: mol_type = other DNA
acacgtgggtattccacagc

SEQ ID NO: 47 - DNA, 20 bp, synthetic construct
  misc_feature 1..20: note = source = /note="Description of Artificial Sequence: Synthetic primer"
  source 1..20: mol_type = other DNA
gtggatcttcagtggtggca

SEQ ID NO: 48 - DNA, 20 bp, synthetic construct
  misc_feature 1..20: note = source = /note="Description of Artificial Sequence: Synthetic primer"
  source 1..20: mol_type = other DNA
atgctccctcatcctttgca

SEQ ID NO: 49 - DNA, 20 bp, synthetic construct
  misc_feature 1..20: note = source = /note="Description of Artificial Sequence: Synthetic primer"
  source 1..20: mol_type = other DNA
agcctctgaacttgactgcc

SEQ ID NO: 50 - DNA, 20 bp, synthetic construct
  misc_feature 1..20: note = source = /note="Description of Artificial Sequence: Synthetic primer"
  source 1..20: mol_type = other DNA
gcctggaactcctgacagtc

SEQ ID NO: 51 - DNA, 20 bp, synthetic construct
  misc_feature 1..20: note = source = /note="Description of Artificial Sequence: Synthetic primer"
  source 1..20: mol_type = other DNA
ggtccttgatccacccagac

SEQ ID NO: 52 - DNA, 20 bp, synthetic construct
  misc_feature 1..20: note = source = /note="Description of Artificial Sequence: Synthetic primer"
  source 1..20: mol_type = other DNA
acatggtgctggtctaaccg

SEQ ID NO: 53 - DNA, 23 bp, synthetic construct
  misc_feature 1..23: note = source = /note="Description of Artificial Sequence: Synthetic primer"
  source 1..23: mol_type = other DNA
catcgagcatcaaatgaaactgc

SEQ ID NO: 54 - DNA, 22 bp, synthetic construct
  misc_feature 1..22: note = source = /note="Description of Artificial Sequence: Synthetic primer"
  source 1..22: mol_type = other DNA
acgttatacgatgtcgcagagt

SEQ ID NO: 55 - DNA, 22 bp, synthetic construct
  misc_feature 1..22: note = source = /note="Description of Artificial Sequence: Synthetic primer"
  source 1..22: mol_type = other DNA
aggcaactttatgcccatgcaa

SEQ ID NO: 56 - DNA, 24 bp, synthetic construct
  misc_feature 1..24: note = source = /note="Description of Artificial Sequence: Synthetic primer"
  source 1..24: mol_type = other DNA
ccaaggggttatgctagttattgc

SEQ ID NO: 57 - DNA, 11 bp, synthetic construct
  misc_feature 1..11: note = source = /note="Description of Artificial Sequence: Synthetic oligonucleotide"
  source 1..11: mol_type = other DNA
tcgaccggatc

SEQ ID NO: 58 - DNA, 11 bp, synthetic construct
  misc_feature 1..11: note = source = /note="Description of Artificial Sequence: Synthetic oligonucleotide"
  misc_feature 1..11: note = source = /note="Description of Combined DNA/RNA Molecule: Synthetic oligonucleotide"
  source 1..11: mol_type = other DNA
  misc_feature 6: note = RNA
tcgactggatc

SEQ ID NO: 59 - DNA, 13 bp, synthetic construct
  misc_feature 1..13: note = source = /note="Description of Artificial Sequence: Synthetic oligonucleotide"
  source 1..13: mol_type = other DNA
gtcgaccggatcc

SEQ ID NO: 60 - DNA, 13 bp, synthetic construct
  misc_feature 1..13: note = source = /note="Description of Artificial Sequence: Synthetic oligonucleotide"
  source 1..13: mol_type = other DNA
gtcgaccggatcc

SEQ ID NO: 61 - DNA, 13 bp, synthetic construct
  misc_feature 1..13: note = source = /note="Description of Artificial Sequence: Synthetic oligonucleotide"
  misc_feature 1..13: note = source = /note="Description of Combined DNA/RNA Molecule: Synthetic oligonucleotide"
  source 1..13: mol_type = other DNA
  misc_feature 13: note = RNA
gtcgaccggatct

SEQ ID NO: 62 - DNA, 11 bp, synthetic construct
  misc_feature 1..11: note = source = /note="Description of Artificial Sequence: Synthetic oligonucleotide"
  source 1..11: mol_type = other DNA
tcgaccggatc

SEQ ID NO: 63 - DNA, 11 bp, synthetic construct
  misc_feature 1..11: note = source = /note="Description of Artificial Sequence: Synthetic oligonucleotide"
  source 1..11: mol_type = other DNA
tcgaccggatc

SEQ ID NO: 64 - DNA, 11 bp, synthetic construct
  misc_feature 1..11: note = source = /note="Description of Artificial Sequence: Synthetic oligonucleotide"
  source 1..11: mol_type = other DNA
tcgaccggatc

SEQ ID NO: 65 - DNA, 11 bp, synthetic construct
  misc_feature 1..11: note = source = /note="Description of Artificial Sequence: Synthetic oligonucleotide"
  source 1..11: mol_type = other DNA
tcgaccggatc

SEQ ID NO: 66 - DNA, 11 bp, synthetic construct
  misc_feature 1..11: note = source = /note="Description of Artificial Sequence: Synthetic oligonucleotide"
  source 1..11: mol_type = other DNA
tcgaccggatc

SEQ ID NO: 67 - DNA, 10 bp, synthetic construct
  misc_feature 1..10: note = source = /note="Description of Artificial Sequence: Synthetic oligonucleotide"
  source 1..10: mol_type = other DNA
cctgtcgagc

SEQ ID NO: 68 - DNA, 10 bp, synthetic construct
  misc_feature 1..10: note = source = /note="Description of Artificial Sequence: Synthetic oligonucleotide"
  source 1..10: mol_type = other DNA
cctgttgagc

SEQ ID NO: 69 - DNA, 10 bp, synthetic construct
  misc_feature 1..10: note = source = /note="Description of Artificial Sequence: Synthetic oligonucleotide"
  source 1..10: mol_type = other DNA
agtcttgatc

SEQ ID NO: 70 - DNA, 10 bp, synthetic construct
  misc_feature 1..10: note = source = /note="Description of Artificial Sequence: Synthetic oligonucleotide"
  source 1..10: mol_type = other DNA
agtctcgatc

SEQ ID NO: 71 - DNA, 119 bp, synthetic construct
  misc_feature 1..119: note = source = /note="Description of Artificial Sequence: Synthetic polynucleotide"
  source 1..119: mol_type = other DNA
atactcatcattaaacttcgcccttacctaccacttcgtgtatgatgataggtagtatacaattgatatcgaaatgagtacgtagatagtagaaagtaagatggaggtgagagtgagag

SEQ ID NO: 72 - DNA, 119 bp, synthetic construct
  misc_feature 1..119: note = source = /note="Description of Artificial Sequence: Synthetic polynucleotide"
  source 1..119: mol_type = other DNA
atactcatcattaaacttcgcccttacctaccacttcgtgtatgtagataggtagtatacaattgatatcgaaatgagtacgtagatagtagaaagtaagatggaggtgagagtgagag

SEQ ID NO: 73 - DNA, 119 bp, synthetic construct
  misc_feature 1..119: note = source = /note="Description of Artificial Sequence: Synthetic polynucleotide"
  source 1..119: mol_type = other DNA
ctctcactctcacctccatcttactttctactatctacgtactcatttcgatatcaattgtatactacctatctacatacacgaagtggtaggtaagggcgaagtttaatgatgagtat

SEQ ID NO: 74 - DNA, 113 bp, synthetic construct
  misc_feature 1..113: note = source = /note="Description of Artificial Sequence: Synthetic polynucleotide"
  source 1..113: mol_type = other DNA
gcgtgatactggtcccgagcctgaagttaggcccgggatgactgacagtcttccgagaccgacgacacaggtctccctatagtgagtcgtattatggcgagagaatgaatctc

SEQ ID NO: 75 - DNA, 113 bp, synthetic construct
  misc_feature 1..113: note = source = /note="Description of Artificial Sequence: Synthetic polynucleotide"
  source 1..113: mol_type = other DNA
gagattcattctctcgccataatacgactcactatagggagacctgtgtcgtcggtctcggaagactgtcagtcatcccgggcctaacttcaggctcgggaccagtatcacgc

SEQ ID NO: 76 - DNA, 10 bp, synthetic construct
  misc_feature 1..10: note = source = /note="Description of Artificial Sequence: Synthetic oligonucleotide"
  source 1..10: mol_type = other DNA
cctgtcgagc